European Patent Specification EP 3 592 374 B1, published February 28, 2024. Title: BACILLUS AMYLOLIQUEFACIENS GF423 STRAIN, AND COMPOSITION FOR PROVIDING ANTIOXIDANT AND ANTI-INFLAMMATORY ACTIVITIES OR PREVENTING OR TREATING HYPERLIPIDEMIA, INCLUDING POLYPEPTIDE PRODUCED BY THE SAME. Applicant: GENOFOCUS, INC. The sequence listing filed with the application follows.

SEQUENCE LISTING (11 sequences)

SEQ ID NO: 1 - DNA, 606 bp, Bacillus amyloliquefaciens
atggcttacaaacttccagaattgccttacgcttatgatgctttagaacctcatatcgataaggaaacgatgacgattcaccatacgaagcaccataacacatacgtgacaaacctcaacaaagcgatcgaaggatctgcgcttgcagagaaatctgtagatgagcttgttgctgatttgaacgcagtgccggaggacatccgcacggcagtccgcaacaatggcggcggacatgcaaaccactctttattctggactcttttatctccgaacggcggaggcgaaccgactggtgagcttgctgaagagatcaaaagcacgttcggaagcttcgatcaatttaaagaaaaattcgccgcagcagctgcaggccgtttcggttcaggctgggcttggctcgttgtaaacaacggcaaacttgaaattacaagcacgccaaaccaagattcaccgctttcagaaggtaaaacacctgttctcggtcttgatgtttgggagcatgcgtactacctgaactaccaaaaccgccgtcctgattacatttcagctttctggaatgttgtgaactgggatgaagttgcccgtctttacagcgaagcaaaataa

SEQ ID NO: 2 - protein, 201 aa, Bacillus amyloliquefaciens
MAYKLPELPYAYDALEPHIDKETMTIHHTKHHNTYVTNLNKAIEGSALAEKSVDELVADLNAVPEDIRTAVRNNGGGHANHSLFWTLLSPNGGGEPTGELAEEIKSTFGSFDQFKEKFAAAAAGRFGSGWAWLVVNNGKLEITSTPNQDSPLSEGKTPVLGLDVWEHAYYLNYQNRRPDYISAFWNVVNWDEVARLYSEAK

SEQ ID NO: 3 - DNA, 1543 bp, Bacillus amyloliquefaciens
agagtttgatcctggctcaggacgaacgctggcggcgtgcctaatacatgcaagtcgagcggacagatgggagcttgctccctgatgtcagcggcggacgggtgagtaacacgtgggtaacctgcctgtaagactgggataactccgggaaaccggggctaataccggatggttgtttgaaccgcatggttcagacataaaaggtggcttcggctaccacttacagatggacccgcggcgcattagctagttggtgaggtaacggctcaccaaggcaacgatgcgtagccgacctgagagggtgatcggccacactgggactgagacacggcccagactcctacgggaggcagcagtagggaatcttccgcaatggacgaaagtctgacggagcaacgccgcgtgagtgatgaaggttttcggatcgtaaagctctgttgttagggaagaacaagtgccgttcaaatagggcggcaccttgacggtacctaaccagaaagccacggctaactacgtgccagcagccgcggtaatacgtaggtggcaagcgttgtccggaattattgggcgtaaagggctcgcaggcggtttcttaagtctgatgtgaaagcccccggctcaaccggggagggtcattggaaactggggaacttgagtgcagaagaggagagtggaattccacgtgtagcggtgaaatgcgtagagatgtggaggaacaccagtggcgaaggcgactctctggtctgtaactgacgctgaggagcgaaagcgtggggagcgaacaggattagataccctggtagtccacgccgtaaacgatgagtgctaagtgttagggggtttccgccccttagtgctgcagctaacgcattaagcactccgcctggggagtacggtcgcaagactgaaactcaaaggaattgacgggggcccgcacaagcggtggagcatgtggtttaattcgaagcaacgcgaagaaccttaccaggtcttgacatcctctgacaatcctagagataggacgtccccttcgggggcagagtgacaggtggtgcatggttgtcgtcagctcgtgtcgtgagatgttgggttaagtcccgcaacgagcgcaacccttgatcttagttgccagcattcagttgggcactctaaggtgactgccggtgacaaaccggaggaaggtggggatgacgtcaaatcatcatgccccttatgacctgggctacacacgtgctacaatggacagaacaaagggcagcgaaaccgcgaggttaagccaatcccacaaatctgttctcagttcggatcgcagtctgcaactcgactgcgtgaagctggaatcgctagtaatcgcggatcagcatgccgcggtgaatacgttcccgggccttgtacacaccgcccgtcacaccacgagagtttgtaacacccgaagtcggtgaggtaacctttatggagccagccgccgaaggtgggacagatgattggggtgaagtcgtaacaaggtagccgtatcggaaggtgcggctggatcacctccttt

SEQ ID NO: 4 - DNA, 1543 bp, Bacillus amyloliquefaciens
agagtttgatcctggctcaggacgaacgctggcggcgtgcctaatacatgcaagtcgagcggacagatgggagcttgctccctgatgttagcggcggacgggtgagtaacacgtgggtaacctgcctgtaagactgggataactccgggaaaccggggctaatagcggatggttgtttgaaccgcatggttcagacataaaaggtggcttcggctaccacttacagatggacccgcggcgcattagctagttggtgaggtaacggctcaccaaggcgacgatgcgtagccgacctgagagggtgatcggccacactgggactgagacacggcccagactcctacgggaggcagcagtagggaatcttccgcaatggacgaaagtctgacggagcaacgccgcgtgagtgatgaaggttttcggatcgtaaagctctgttgttagggaagaacaagtgccgttcaaatagggcggcaccttgacggtacctaaccagaaagccacggctaactacgtgccagcagccgcggtaatacgtaggtggcaagcgttgtccggaattattgggcgtaaagggctcgcaggcggtttcttaagtctgatgtgaaagcccccggctcaaccggggagggtcattggaaactggggaacttgagtgcagaagaggagagtggaattccacgtgtagcggtgaaatgcgtagagatgtggaggaacaccagtggcgaaggcgactctctggtctgtaactgacgctgaggagcgaaagcgtggggagcgaacaggattagataccctggtagtccacgccgtaaacgatgagtgctaagtgttagggggtttccgccccttagtgctgcagctaacgcattaagcactccgcctggggagtacggtcgcaagactgaaactcaaaggaattgacgggggcccgcacaagcggtggagcatgtggtttaattcgaagcaacgcgaagaaccttaccaggtcttgacatcctctgacaatcctagagataggacgtccccttcgggggcagagtgacaggtggtgcatggttgtcgtcagctcgtgtcgtgagatgttgggttaagtcccgcaacgagcgcaacccttgatcttagttgccagcattcagttgggcactctaaggtgactgccggtgacaaaccggaggaaggtggggatgacgtcaaatcatcatgccccttatgacctgggctacacacgtgctacaatggacagaacaaagggcagcgaaaccgcgaggttaagccaatcccacaaatctgttctcagttcggatcgcagtctgcaactcgactgcgtgaagctggaatcgctagtaatcgcggatcagcatgccgcggtgaatacgttcccgggccttgtacacaccgcccgtcacaccacgagagtttgtaacacccgaagtcggtgaggtaacctttatggagccagccgccgaaggtgggacagatgattggggtgaagtcgtaacaaggtagccgtatcggaaggtgcggctggatcacctccttt

SEQ ID NO: 5 - DNA, 1543 bp, Bacillus amyloliquefaciens
agagtttgatcctggctcaggacgaacgctggcggcgtgcctaatacatgcaagtcgagcggacagatgggagcttgctccctgatgttagcggcggacgggtgagtaacacgtgggtaacctgcctgtaagactgggataactccgggaaaccggggctaataccggatggttgtctgaaccgcatggttcagacataaaaggtggcttcggctaccacttacagatggacccgcggcgcattagctagttggtgaggtaacggctcaccaaggcgacgatgcgtagccgacctgagagggtgatcggccacactgggactgagacacggcccagactcctacgggaggcagcagtagggaatcttccgcaatggacgaaagtctgacggagcaacgccgcgtgagtgatgaaggttttcggatcgtaaagctctgttgttagggaagaacaagtgccgttcaaatagggcggcaccttgacggtacctaaccagaaagccacggctaactacgtgccagcagccgcggtaatacgtaggtggcaagcgttgtccggaattattgggcgtaaagggctcgcaggcggtttcttaagtctgatgtgaaagcccccggctcaaccggggagggtcattggaaactggggaacttgagtgcagaagaggagagtggaattccacgtgtagcggtgaaatgcgtagagatgtggaggaacaccagtggcgaaggcgactctctggtctgtaactgacgctgaggagcgaaagcgtggggagcgaacaggattagataccctggtagtccacgccgtaaacgatgagtgctaagtgttagggggtttccgccccttagtgctgcagctaacgcattaagcactccgcctggggagtacggtcgcaagactgaaactcaaaggaattgacgggggcccgcacaagcggtggagcatgtggtttaattcgaagcaacgcgaagaaccttaccaggtcttgacatcctctgacaatcctagagataggacgtccccttcgggggcagagtgacaggtggtgcatggttgtcgtcagctcgtgtcgtgagatgttgggttaagtcccgcaacgagcgcaacccttgatcttagttgccagcattcagttgggcactctaaggtgactgccggtgacaaaccggaggaaggtggggatgacgtcaaatcatcatgccccttatgacctgggctacacacgtgctacaatggacagaacaaagggcagcgaaaccgcgaggttaagccaatcccacaaatctgttctcagttcggatcgcagtctgcaactcgactgcgtgaagctggaatcgctagtaatcgcggatcagcatgccgcggtgaatacgttcccgggccttgtacacaccgcccgtcacaccacgagagtttgtaacacccgaagtcggtgaggtaacctttatggagccagccgccgaaggtgggacagatgattggggtgaagtcgtaacaaggtagccgtatcggaaggtgcggctggatcacctccttt

SEQ ID NO: 6 - DNA, 1543 bp, Bacillus amyloliquefaciens
agagtttgatcctggctcaggacgaacgctggcggcgtgcctaatacatgcaagtcgagcggacagatgggagcttgctccctgatgttagcggcggacgggtgagtaacacgtgggtaacctgcctgtaagactgggataactccgggaaaccggggctaataccggatggttgtttgaaccgcatggttcagacataaaaggtggcttcggctaccacttacagatggacccgcggcgcattagctagttggtgaggtaacggctcaccaaggcgacgatgcgtagccgacctgagagggtgatcggccacactgggactgagacacggcccagactcctacgggaggcagcagtagggaatcttccgcaatggacgaaagtctgacggagcaacgccgcgtgagtgatgaaggttttcggatcgtaaagctctgttgttagggaagaacaagtgccgttcaaatagggcggcaccttgacggtacctaaccagaaagccacggctaactacgtgccagcagccgcggtaatacgtaggtggcaagcgttgtccggaattattgggcgtaaagggctcgcaggcggtttcttaagtctgatgtgaaagcccccggctcaaccggggagggtcattggaaactggggaacttgagtgcagaagaggagagtggaattccacgtgtagcggtgaaatgcgtagagatgtggaggaacaccagtggcgaaggcgactctctggtctgtaactgacgctgaggagcgaaagcgtggggagcgaacaggattagataccctggtagtccacgccgtaaacgatgagtgctaagtgttagggggtttccgccccttagtgctgcagctaacgcattaagcactccgcctggggagtacggtcgcaagactgaaactcaaaggaattgacgggggcccgcacaagcggtggagcatgtggtttaattcgaagcaacgcgaagaaccttaccaggtcttgacatcctctgacaatcctagagataggacgtccccttcgggggcagagtgacaggtggtgcatggttgtcgtcagctcgtgtcgtgagatgttgggttaagtcccgcaacgagcgcaacccttgatcttagttgccagcattcagttgggcactctaaggtgactgccggtgacaaaccggaggaaggtggggatgacgtcaaatcatcatgccccttatgacctgggctacacacgtgctacaatggacagaacaaagggcagcgaaaccgcgaggttaagccaatcccacaaatctgttctcagttcggatcgcagtctgcaactcgactgcgtgaagctggaatcgctagtaatcgcggatcagcatgccgcggtgaatacgttcccgggccttgtacacaccgcccgtcacaccacgagagtttgtaacacccgaagtcggtgaggtaacctttatggagccagccgccgaaggtgggacagatgattggggtgaagtcgtaacaaggtagccgtatcggaaggtgcggctggatcacctccttt

SEQ ID NO: 7 - DNA, 1543 bp, Bacillus amyloliquefaciens
agagtttgatcctggctcaggacgaacgctggcggcgtgcctaatacatgcaagtcgagcggacagatgggagcttgctccctgatgttagcggcggacgggtgagtaacacgtgggtaacctgcctgtaagactgggataactccgggaaaccggggctaataccggatggttgtctgaaccgcatggttcagacataaaaggtggcttcggctaccacttacagatggacccgcggcgcattagctagttggtgaggtaacggctcaccaaggcgacgatgcgtagccgacctgagagggtgatcggccacactgggactgagacacggcccagactcctacgggaggcagcagtagggaatcttccgcaatggacgaaagtctgacggagcaacgccgcgtgagtgatgaaggttttcggatcgtaaagctctgttgttagggaagaacaagtgccgttcaaatagggcggcaccttgacggtacctaaccagaaagccacggctaactacgtgccagcagccgcggtaatacgtaggtggcaagcgttgtccggaattattgggcgtaaagggctcgcaggcggtttcttaagtctgatgtgaaagcccccggctcaaccggggagggtcattggaaactggggaacttgagtgcagaagaggagagtggaattccacgtgtagcggtgaaatgcgtagagatgtggaggaacaccagtggcgaaggcgactctctggtctgtaactgacgctgaggagcgaaagcgtggggagcgaacaggattagataccctggtagtccacgccgtaaacgatgagtgctaagtgttagggggtttccgccccttagtgctgcagctaacgcattaagcactccgcctggggagtacggtcgcaagactgaaactcaaaggaattgacgggggcccgcacaagcggtggagcatgtggtttaattcgaagcaacgcgaagaaccttaccaggtcttgacatcctctgacaatcctagagataggatgtccccttcgggggcagagtgacaggtggtgcatggttgtcgtcagctcgtgtcgtgagatgttgggttaagtcccgcaacgagcgcaacccttgatcttagttgccagcattcagttgggcactctaaggtgactgccggtgacaaaccggaggaaggtggggatgacgtcaaatcatcatgccccttatgacctgggctacacacgtgctacaatggacagaacaaagggcagcgaaaccgcgaggttaagccaatcccacaaatctgttctcagttcggatcgcagtctgcaactcgactgcgtgaagctggaatcgctagtaatcgcggatcagcatgccgcggtgaatacgttcccgggccttgtacacaccgcccgtcacaccacgagagtttgtaacacccgaagtcggtgaggtaacctttatggagccagccgccgaaggtgggacagatgattggggtgaagtcgtaacaaggtagccgtatcggaaggtgcggctggatcacctccttt

SEQ ID NO: 8 - DNA, 1543 bp, Bacillus amyloliquefaciens; identical to SEQ ID NO: 7

SEQ ID NO: 9 - DNA, 1543 bp, Bacillus amyloliquefaciens
agagtttgatcctggctcaggacgaacgctggcggcgtgcctaatacatgcaagtcgagcggacagatgggagcttgctccctgatgttagcggcggacgggtgagtaacacgtgggtaacctgcctgtaagactgggataactccgggaaaccggggctaataccggatggttgtttgaaccgcatggttcagacataaaaggtggcttcggctaccacttacagatggacccgcggcgcattagctagttggtgaggtaacggctcaccaaggcaacgatgcgtagccgacctgagagggtgatcggccacactgggactgagacacggcccagactcctacgggaggcagcagtagggaatcttccgcaatggacgaaagtctgacggagcaacgccgcgtgagtgatgaaggttttcggatcgtaaagctctgttgttagggaagaacaagtgccgttcaaatagggcggcaccttgacggtacctaaccagaaagccacggctaactacgtgccagcagccgcggtaatacgtaggtggcaagcgttgtccggaattattgggcgtaaagggctcgcaggcggtttcttaagtctgatgtgaaagcccccggctcaaccggggagggtcattggaaactggggaacttgagtgcagaagaggagagtggaattccacgtgtagcggtgaaatgcgtagagatgtggaggaacaccagtggcgaaggcgactctctggtctgtaactgacgctgaggagcgaaagcgtggggagcgaacaggattagataccctggtagtccacgccgtaaacgatgagtgctaagtgttagggggtttccgccccttagtgctgcagctaacgcattaagcactccgcctggggagtacggtcgcaagactgaaactcaaaggaattgacgggggcccgcacaagcggtggagcatgtggtttaattcgaagcaacgcgaagaaccttaccaggtcttgacatcctctgacaatcctagagataggacgtccccttcgggggcagagtgacaggtggtgcatggttgtcgtcagctcgtgtcgtgagatgttgggttaagtcccgcaacgagcgcaacccttgatcttagttgccagcattcagttgggcactctaaggtgactgccggtgacaaaccggaggaaggtggggatgacgtcaaatcatcatgccccttatgacctgggctacacacgtgctacaatggacagaacaaagggcagcgaaaccgcgaggttaagccaatcccacaaatctgttctcagttcggatcgcagtctgcaactcgactgcgtgaagctggaatcgctagtaatcgcggatcagcatgccgcggtgaatacgttcccgggccttgtacacaccgcccgtcacaccacgagagtttgtaacacccgaagtcggtgaggtaacctttatggagccagccgccgaaggtgggacagatgattggggtgaagtcgtaacaaggtagccgtatcggaaggtgcggctggatcacctccttt

SEQ ID NO: 10 - DNA, 1543 bp, Bacillus amyloliquefaciens
agagtttgatcctggctcaggacgaacgctggcggcgtgcctaatacatgcaagtcgagcggacagatgggagcttgctccctgatgttagcggcggacgggtgagtaacacgtgggtaacctgcctgtaagactgggataactccgggaaaccggggctaataccggatggttgtctgaatcgcatggttcagacataaaaggtggcttctgctaccacttacagatggacccgcggcgcattagctagttggtgaggtaacggctcaccaaggcgacgatgcgtagccgacctgagagggtgatcggccacactgggactgagacacggcccagactcctacgggaggcagcagtagggaatcttccgcaatggacgaaagtctgacggagcaacgccgcgtgagtgatgaaggttttcggatcgtaaagctctgttgttagggaagaacaagtgccgttcaaatagggcggcaccttgacggtacctaaccagaaagccacggctaactacgtgccagcagccgcggtaatacgtaggtggcaagcgttgtccggaattattgggcgtaaagggctcgcaggcggtttcttaagtctgatgtgaaagcccccggctcaaccggggagggtcattggaaactggggaacttgagtgcagaagaggagagtggaattccacgtgtagcggtgaaatgcgtagagatgtggaggaacaccagtggcgaaggcgactctctggtctgtaactgacgctgaggagcgaaagcgtggggagcgaacaggattagataccctggtagtccacgccgtaaacgatgagtgctaagtgttagggggtttccgccccttagtgctgcagctaacgcattaagcactccgcctggggagtacggtcgcaagactgaaactcaaaggaattgacgggggcccgcacaagcggtggagcatgtggtttaattcgaagcaacgcgaagaaccttaccaggtcttgacatcctctgacaatcctagagataggacgtccccttcgggggcagagtgacaggtggtgcatggttgtcgtcagctcgtgtcgtgagatgttgggttaagtcccgcaacgagcgcaacccttgatcttagttgccagcattcagttgggcactctaaggtgactgccggtgacaaaccggaggaaggtggggatgacgtcaaatcatcatgccccttatgacctgggctacacacgtgctacaatggacagaacaaagggcagcgaaaccgcgaggttaagccaatcccacaaatctgttctcagttcggatcgcagtctgcaactcgactgcgtgaagctggaatcgctagtaatcgcggatcagcatgccgcggtgaatacgttcccgggccttgtacacaccgcccgtcacaccacgagagtttgtaacacccgaagtcggtgaggtaaccttttaggagccagccgccgaaggtgggacagatgattggggtgaagtcgtaacaaggtagccgtatcggaaggtgcggctggatcacctccttt

SEQ ID NO: 11 - DNA, 1543 bp, Bacillus amyloliquefaciens
agagtttgatcctggctcaggacgaacgctggcggcgtgcctaatacatgcaagtcgagcggacagatgggagcttgctccctgatgttagcggcggacgggtgagtaacacgtgggtaacctgcctgtaagactgggataactccgggaaaccggggctaataccagatggttgtctgaaccgcatggttcagacataaaaggtggcttcggctaccacttacagatggacccgcggcgcattagctagttggtgaggtaacggctcaccaaggcgacgatgcgtagccgacctgagagggtgatcggccacactgggactgagacacggcccagactcctacgggaggcagcagtagggaatcttccgcaatggacgaaagtctgacggagcaacgccgcgtgagtgatgaaggttttcggatcgtaaagctctgttgttagggaagaacaagtgccgttcaaatagggcggcaccttgacggtacctaaccagaaagccacggctaactacgtgccagcagccgcggtaatacgtaggtggcaagcgttgtccggaattattgggcgtaaagggctcgcaggcggtttcttaagtctgatgtgaaagcccccggctcaaccggggagggtcattggaaactggggaacttgagtgcagaagaggagagtggaattccacgtgtagcggtgaaatgcgtagagatgtggaggaacaccagtggcgaaggcgactctctggtctgtaactgacgctgaggagcgaaagcgtggggagcgaacaggattagataccctggtagtccacgccgtaaacgatgagtgctaagtgttagggggtttccgccccttagtgctgcagctaacgcattaagcactccgcctggggagtacggtcgcaagactgaaactcaaaggaattgacgggggcccgcacaagcggtggagcatgtggtttaattcgaagcaacgcgaagaaccttaccaggtcttgacatcctctgacaatcctagagataggacgtccccttcgggggcagagtgacaggtggtgcatggttgtcgtcagctcgtgtcgtgagatgttgggttaagtcccgcaacgagcgcaacccttgatcttagttgccagcattcagttgggcactctaaggtgactgccggtgacaaaccggaggaaggtggggatgacgtcaaatcatcatgccccttatgacctgggctacacacgtgctacaatggacagaacaaagggcagcgaaaccgcgaggttaagccaatcccacaaatctgttctcagttcggatcgcagtctgcaactcgactgcgtgaagctggaatcgctagtaatcgcggatcagcatgccgcggtgaatacgttcccgggccttgtacacaccgcccgtcacaccacgagagtttgtaacacccgaagtcggtgaggtaaccttttaggagccagccgccgaaggtgggacagatgattggggtgaagtcgtaacaaggtagccgtatcggaaggtgcggctggatcacctccttt